European Patent Specification EP 3 936 188 B1, published November 29, 2023. Title: VECTORS AND METHODS FOR REGENERATIVE THERAPY. Applicant: UNIVERSITY OF WASHINGTON. The sequence listing filed with the application follows.

SEQUENCE LISTING (54 sequences)

SEQ ID NO: 1 - protein, 523 aa, Homo sapiens [sequence omitted]

SEQ ID NO: 2 - protein, 31 aa, Artificial Sequence
  FLAG and  MYC tags
  myc (7)..(16): myc tag
  flag (23)..(30): flag tag
TRTLPLEQKLISEEDLAANDILDYKDDDDKV

SEQ ID NO: 3 - DNA, 22 bp, Artificial Sequence
  primer
ccaatgtgtccgtcgtggatct

SEQ ID NO: 4 - DNA, 22 bp, Artificial Sequence
  primer
gttgaagtcgcaggagacaacc

SEQ ID NO: 5 - DNA, 21 bp, Artificial Sequence
  primer
aggattggagcccagagtgga

SEQ ID NO: 6 - DNA, 21 bp, Artificial Sequence
  primer
tgatagatgaaggcaggaagc

SEQ ID NO: 7 - DNA, 23 bp, Artificial Sequence
  primer
gcgactcaaaaagaaggactttg

SEQ ID NO: 8 - DNA, 20 bp, Artificial Sequence
  primer
ggcttgctcatcctcaatcc

SEQ ID NO: 9 - DNA, 20 bp, Artificial Sequence
  primer
agaagcccagcgctccctca

SEQ ID NO: 10 - DNA, 20 bp, Artificial Sequence
  primer
gggcgttcttggccttgcct

SEQ ID NO: 11 - DNA, 22 bp, Artificial Sequence
  primer
gcagcccagaggaaacccaacc

SEQ ID NO: 12 - DNA, 21 bp, Artificial Sequence
  primer
agccgcatcgctgctctcatc

SEQ ID NO: 13 - DNA, 24 bp, Artificial Sequence
  primer
tgctgcaaatggaactgcttctgg

SEQ ID NO: 14 - DNA, 24 bp, Artificial Sequence
  primer
taccatggagggtgggttggaaat

SEQ ID NO: 15 - DNA, 20 bp, Artificial Sequence
  primer
gcttcgggtctgagttccaa

SEQ ID NO: 16 - DNA, 19 bp, Artificial Sequence
  primer
ggatgaagagcaggggtcc

SEQ ID NO: 17 - DNA, 20 bp, Artificial Sequence
  primer
gggacctgaagccagagaac

SEQ ID NO: 18 - DNA, 20 bp, Artificial Sequence
  primer
ccacagaagagaggcttccg

SEQ ID NO: 19 - DNA, 21 bp, Artificial Sequence
  primer
gcctcacaaagcacatgactg

SEQ ID NO: 20 - DNA, 20 bp, Artificial Sequence
  primer
tcgacaacttccgttagcct

SEQ ID NO: 21 - DNA, 23 bp, Artificial Sequence
  primer
ggcgagttcttcacagagacttg

SEQ ID NO: 22 - DNA, 24 bp, Artificial Sequence
  primer
ccctatactccagatgtcaaccgg

SEQ ID NO: 23 - DNA, 21 bp, Artificial Sequence
  primer
gcacctgaaacatcccaacat

SEQ ID NO: 24 - DNA, 20 bp, Artificial Sequence
  primer
ggtccgactcttctgcagtt

SEQ ID NO: 25 - DNA, 19 bp, Artificial Sequence
  primer
gtattcccaagcacatcaa

SEQ ID NO: 26 - DNA, 19 bp, Artificial Sequence
  primer
gtagccagaagtgaagaac

SEQ ID NO: 27 - DNA, 21 bp, Artificial Sequence
  primer
tgccaagaagtccaagaatca

SEQ ID NO: 28 - DNA, 18 bp, Artificial Sequence
  primer
ctgctgctcactctcctg

SEQ ID NO: 29 - DNA, 18 bp, Artificial Sequence
  primer
tgtccttggcagcactca

SEQ ID NO: 30 - DNA, 22 bp, Artificial Sequence
  primer
ttcaccactgtccttgttctca

SEQ ID NO: 31 - DNA, 24 bp, Artificial Sequence
  primer
cctgataaccttgaacctgcttgt

SEQ ID NO: 32 - DNA, 19 bp, Artificial Sequence
  primer
gctgaggctgcttgtgtct

SEQ ID NO: 33 - DNA, 21 bp, Artificial Sequence
  primer
caccgaacttatgatggacag

SEQ ID NO: 34 - DNA, 18 bp, Artificial Sequence
  primer
atggcttctgctctcact

SEQ ID NO: 35 - DNA, 21 bp, Artificial Sequence
  primer
gcagaggaggagattggaaca

SEQ ID NO: 36 - DNA, 18 bp, Artificial Sequence
  primer
gctacaggcgtggtgact

SEQ ID NO: 37 - DNA, 21 bp, Artificial Sequence
  primer
gcagaccagcctgacagattt

SEQ ID NO: 38 - DNA, 20 bp, Artificial Sequence
  primer
ctgacccacagcagaagagg

SEQ ID NO: 39 - DNA, 20 bp, Artificial Sequence
  primer
cagtgggaaccttctgggac

SEQ ID NO: 40 - DNA, 20 bp, Artificial Sequence
  primer
cgcggatcttgagggtgaaa

SEQ ID NO: 41 - DNA, 20 bp, Artificial Sequence
  primer
ctgctagggctttaggctcc

SEQ ID NO: 42 - DNA, 20 bp, Artificial Sequence
  primer
tttgggaggaacgaccttgg

SEQ ID NO: 43 - DNA, 20 bp, Artificial Sequence
  primer
cagagagcatcacgagcaga

SEQ ID NO: 44 - DNA, 20 bp, Artificial Sequence
  primer
ctcttgggcagctcctcttc

SEQ ID NO: 45 - DNA, 20 bp, Artificial Sequence
  primer
gcgggttcatgcaagttgtt

SEQ ID NO: 46 - DNA, 20 bp, Artificial Sequence
  primer
gtttcagagcacctcccctc

SEQ ID NO: 47 - DNA, 20 bp, Artificial Sequence
  primer
tctgagtctgccttcttctg

SEQ ID NO: 48 - DNA, 22 bp, Artificial Sequence
  primer
gccagggttcacaagtcctgag

SEQ ID NO: 49 - DNA, 20 bp, Artificial Sequence
  primer
ttgatggacaagcctgtacc

SEQ ID NO: 50 - DNA, 20 bp, Artificial Sequence
  primer
tcatttgctgccagatcctc

SEQ ID NO: 51 - DNA, 20 bp, Artificial Sequence
  primer
cctcaacgaccactttgtca

SEQ ID NO: 52 - DNA, 20 bp, Artificial Sequence
  primer
ttactccttggaggccatgt

SEQ ID NO: 53 - DNA, 20 bp, Artificial Sequence
  primer
aagcccagctcaactccatc

SEQ ID NO: 54 - DNA, 20 bp, Artificial Sequence
  primer
tgtccatcaaagccccatcc